European Patent Application EP 4 644 407 A1, published November 5, 2025. Title: Novel porin BCP34, and mutant thereof and use thereof. Applicant: BGI SHENZHEN. Application WO. The sequence listing filed with the application follows.

SEQUENCE LISTING (10 sequences)

SEQ ID NO: 1 - protein, 277 aa, unidentified
MKRFIAFAVSMTLVGCASFSPPKGQTSIRDRAQPLSATVTRNALTKLPPPLAPIPAAVYNIKDQTGQYKPSPSNGFSTAVMQGATSVLVKALLDSRWFIPLEREGLQNLLTERKIIRARDSKKDLSNLAAASVIIEGSIIAYDSNVRTGGAGAKYLGIGLSEQYREDQVTVNLRAINVNNGRILQSVTSTKMIFSRQLDSGAFGYIRFKKLLEIESGYSYNEPAQLCVIDAIESALIQLIYEGVVGGTWKLKNPADIDSPIFTHYAGQNGPEGQAIM

SEQ ID NO: 2 - DNA, 834 bp, unidentified
  source 1..834: mol_type = genomic DNA
atgaagcgctttattgcctttgcagttagcatgaccctggttggttgtgcaagctttagcccgccgaaaggtcagaccagcattcgtgatcgtgcacagcctctgagtgcaaccgttacccgtaatgcactgaccaaactgcctcctcctctggcacctattccggcagcagtttacaatatcaaggatcagaccggtcagtataaaccgagccctagtaatggttttagcaccgcagttatgcagggtgcaaccagcgttctggttaaagcattactggatagccgttggtttattccgctggaacgtgaaggtctgcagaatctgctgaccgaacgcaaaattattcgtgcacgcgacagcaaaaaagatctgagcaatctggcagcagcaagcgttattattgagggtagcatcatcgcctatgatagcaatgttcgtaccggtggtgcaggtgcaaaatatctgggtattggtctgagcgaacagtatcgtgaagatcaggttaccgttaatctgcgcgcaatcaatgttaacaacggccgtattctgcagagcgttaccagcaccaaaatgatttttagccgtcagctggatagcggtgcatttggttatattcgcttcaagaagctgctggagattgaaagcggttacagctataatgaaccggcacagctgtgtgttattgatgcaattgagagcgcactgattcagctgatttatgagggtgttgttggtggtacctggaaactgaaaaatccggccgatattgatagcccgatctttacccattatgccggtcagaatggtcctgaaggtcaggcaattatgtaa

SEQ ID NO: 3 - protein, 277 aa, synthetic construct
MKRFIAFAVSMTLVGCASFSPPKGQTSIRDRAQPLSATVTRNALTKLPPPLAPIPAAVYNIKDQTGQYKPSPSSNASTAVMQGATSVLVKALLDSRWFIPLEREGLQNLLTERKIIRARDSKKDLSNLAAASVIIEGSIIAYDSNVRTGGAGAKYLGIGLSEQYREDQVTVNLRAINVNNGRILQSVTSTKMIFSRQLDSGAFGYIRFKKLLEIESGYSYNEPAQLCVIDAIESALIQLIYEGVVGGTWKLKNPADIDSPIFTHYAGQNGPEGQAIM

SEQ ID NO: 4 - DNA, 834 bp, synthetic construct
  source 1..834: mol_type = other DNA
atgaagcgctttattgcctttgcagttagcatgaccctggttggttgtgcaagctttagcccgccgaaaggtcagaccagcattcgtgatcgtgcacagcctctgagtgcaaccgttacccgtaatgcactgaccaaactgcctcctcctctggcacctattccggcagcagtttacaatatcaaggatcagaccggtcagtataaaccggcaccggcaagcaatcagagcaccgcagttatgcagggtgcaaccagcgttctggttaaagcattactggatagccgttggtttattccgctggaacgtgaaggtctgcagaatctgctgaccgaacgcaaaattattcgtgcacgcgacagcaaaaaagatctgagcaatctggcagcagcaagcgttattattgagggtagcatcatcgcctatgatagcaatgttcgtaccggtggtgcaggtgcaaaatatctgggtattggtctgagcgaacagtatcgtgaagatcaggttaccgttaatctgcgcgcaatcaatgttaacaacggccgtattctgcagagcgttaccagcaccaaaatgatttttagccgtcagctggatagcggtgcatttggttatattcgcttcaagaagctgctggagattgaaagcggttacagctataatgaaccggcacagctgtgtgttattgatgcaattgagagcgcactgattcagctgatttatgagggtgttgttggtggtacctggaaactgaaaaatccggccgatattgatagcccgatctttacccattatgccggtcagaatggtcctgaaggtcaggcaattatgtaa

SEQ ID NO: 5 - DNA, 72 bp, synthetic construct
  source 1..72: mol_type = other DNA
ttttttttttttttttttttttttttttttttttttttttyyyyggttgtttctgttggtgctgatattgct

SEQ ID NO: 6 - DNA, 45 bp, synthetic construct
  source 1..45: mol_type = other DNA
gcaatatcagcaccaacagaaacaacctttgaggcgagcggtcaa

SEQ ID NO: 7 - DNA, 2710 bp, synthetic construct
  source 1..2710: mol_type = other DNA
tcgcgcgtttcggtgatgacggtgaaaacctctgacacatgcagctcccggagacggtcacagcttgtctgtaagcggatgccgggagcagacaagcccgtcagggcgcgtcagcgggtgttggcgggtgtcggggctggcttaactatgcggcatcagagcagattgtactgagagtgcaccatatgcggtgtgaaataccgcacagatgcgtaaggagaaaataccgcatcaggcgccattcgccattcaggctgcgcaactgttgggaagggcgatcggtgcgggcctcttcgctattacgccagctggcgaaagggggatgtgctgcaaggcgattaagttgggtaacgccagggttttcccagtcacgacgttgtaaaacgacggccagtgaattcgagctcggtacctcgcgaatgcatctagatatcggatcccgggcccgtcgactgcagaggcctgcatgcaagcttggcgtaatcatggtcatagctgtttcctgtgtgaaattgttatccgctcacaattccacacaacatacgagccggaagcataaagtgtaaagcctggggtgcctaatgagtgagctaactcacattaattgcgttgcgctcactgcccgctttccagtcgggaaacctgtcgtgccagctgcattaatgaatcggccaacgcgcggggagaggcggtttgcgtattgggcgctcttccgcttcctcgctcactgactcgctgcgctcggtcgttcggctgcggcgagcggtatcagctcactcaaaggcggtaatacggttatccacagaatcaggggataacgcaggaaagaacatgtgagcaaaaggccagcaaaaggccaggaaccgtaaaaaggccgcgttgctggcgtttttccataggctccgcccccctgacgagcatcacaaaaatcgacgctcaagtcagaggtggcgaaacccgacaggactataaagataccaggcgtttccccctggaagctccctcgtgcgctctcctgttccgaccctgccgcttaccggatacctgtccgcctttctcccttcgggaagcgtggcgctttctcatagctcacgctgtaggtatctcagttcggtgtaggtcgttcgctccaagctgggctgtgtgcacgaaccccccgttcagcccgaccgctgcgccttatccggtaactatcgtcttgagtccaacccggtaagacacgacttatcgccactggcagcagccactggtaacaggattagcagagcgaggtatgtaggcggtgctacagagttcttgaagtggtggcctaactacggctacactagaagaacagtatttggtatctgcgctctgctgaagccagttaccttcggaaaaagagttggtagctcttgatccggcaaacaaaccaccgctggtagcggtggtttttttgtttgcaagcagcagattacgcgcagaaaaaaaggatctcaagaagatcctttgatcttttctacggggtctgacgctcagtggaacgaaaactcacgttaagggattttggtcatgagattatcaaaaaggatcttcacctagatccttttaaattaaaaatgaagttttaaatcaatctaaagtatatatgagtaaacttggtctgacagttaccaatgcttaatcagtgaggcacctatctcagcgatctgtctatttcgttcatccatagttgcctgactccccgtcgtgtagataactacgatacgggagggcttaccatctggccccagtgctgcaatgataccgcgagacccacgctcaccggctccagatttatcagcaataaaccagccagccggaagggccgagcgcagaagtggtcctgcaactttatccgcctccatccagtctattaattgttgccgggaagctagagtaagtagttcgccagttaatagtttgcgcaacgttgttgccattgctacaggcatcgtggtgtcacgctcgtcgtttggtatggcttcattcagctccggttcccaacgatcaaggcgagttacatgatcccccatgttgtgcaaaaaagcggttagctccttcggtcctccgatcgttgtcagaagtaagttggccgcagtgttatcactcatggttatggcagcactgcataattctcttactgtcatgccatccgtaagatgcttttctgtgactggtgagtactcaaccaagtcattctgagaatagtgtatgcggcgaccgagttgctcttgcccggcgtcaatacgggataataccgcgccacatagcagaactttaaaagtgctcatcattggaaaacgttcttcggggcgaaaactctcaaggatcttaccgctgttgagatccagttcgatgtaacccactcgtgcacccaactgatcttcagcatcttttactttcaccagcgtttctgggtgagcaaaaacaggaaggcaaaatgccgcaaaaaagggaataagggcgacacggaaatgttgaatactcatactcttcctttttcaatattattgaagcatttatcagggttattgtctcatgagcggatacatatttgaatgtatttagaaaaataaacaaataggggttccgcgcacatttccccgaaaagtgccacctgacgtctaagaaaccattattatcatgacattaacctataaaaataggcgtatcacgaggccctttcgtc

SEQ ID NO: 8 - protein, 454 aa, synthetic construct
MKHDLSSATEEQRYIFTDFIKQAQLALKGDSDYEVFAIQGFAGSGKTWLSALIIDELLELGMKVAVTSPTHKAVRVSLNMLKNNGIDTNSPLMYPGTIHHFLNLKLDHGFADDGTACNVTTKAKLVVNKFNEALEYVDVLIVDEASMVSGELYDHALKTLGDRAKIILFIGDSYQLLPVDDEDSSIFLKDDIFHYKLTKVVRQAEDNIIIAKSQELIKAMDQKTYYPSVNDYFVNITEDTEGIKLLKSNVELFELYFSDFKDKMTGAYTNKVVNQFNEYIRYTLYQETKFIADKDELVFQETYTDSKGNIIVSNGEIIEVATAKLTTDIDKFKIWKIVSKKNELGEAVRFNVLDPSSYNEFNDLLDKYCADAKIAKGYDRSKAWKKYFKLKEKYAKVRYNFSSTIHKLQGSTYQNMYFDMRGLDYFYRMNRDNVLRLVYVGITRASDQVFILQD

SEQ ID NO: 9 - DNA, 15 bp, synthetic construct
  source 1..15: mol_type = other DNA
ttgaccgctcgcctc

SEQ ID NO: 10 - DNA, 24 bp, synthetic construct
  source 1..24: mol_type = other DNA
ttttttttttggtggtgtggttgg